European Patent Application EP 4 461 737 A1, published November 13, 2024. Title: Polypeptide for Delivering Antigen to Immune Cells. Applicant: JW CreaGene Inc. The sequence listing filed with the application follows.

SEQUENCE LISTING (7 sequences)

SEQ ID NO: 1 - protein, 12 aa, synthetic construct
  REGION 1..12: note = SEB1
KSIDQFLYFDLY

SEQ ID NO: 2 - protein, 11 aa, synthetic construct
  REGION 1..11: note = SEB2
IYSIKDTKLGN

SEQ ID NO: 3 - protein, 25 aa, synthetic construct
  REGION 1..25: note = SEB3
YYQCYFSKKTNDINSHQTDKRKTCM

SEQ ID NO: 4 - protein, 12 aa, synthetic construct
  REGION 1..12: note = SEB4
YNKKKATVQELD

SEQ ID NO: 5 - protein, 11 aa, synthetic construct
  REGION 1..11: note = CTP512
YGRRARRRRRR

SEQ ID NO: 6 - protein, 11 aa, synthetic construct
  REGION 1..11: note = CTP509
YKRKARRAARR

SEQ ID NO: 7 - protein, 11 aa, synthetic construct
  REGION 1..11: note = CTP513
YGRRRRRRRRR